European Patent Application EP 4 428 240 A1, published September 11, 2024. Title: Erythritol induced promoter and method of producing a target substance using the same. Applicant: Kao Corporation. The sequence listing filed with the application follows.

SEQUENCE LISTING (26 sequences)

SEQ ID NO: 1 - DNA, 1000 bp, Trichoderma reesei
  source 1..1000: mol_type = genomic DNA
cttcgacatcaaaatcaccttgttctctgtggggggatcgcatgaggaggcgtttgccggcggctagtggctggtctcctccacaaaatgcccttcggaaacaaaacgccagggggccattccaaaagccggctaaccgtcgctggtaatccgaagttcagcgtggcactcccaagctgcaaattgcttctccaaaaaaagcacccatcaattcacactcggtatccggatgaattccagtctgttcagctcgcatttccagcctgggaagagatggagactttccgtcctgaagtccgcccacgccgtttgccatgttcacccctcatcaacctctgccacaccacctttccggggccggaggagctccccggtccaagttgccgagctcttgtagaagcttagctttgctcgcgcttcacgtcgtattgtgctgcacgtctcggcggtcgtctttgattcgatccttcatcgattctcttgccctgctaccacacctcccccaaggccaatcgttcactcccttccccgctcgtccccattgtgcttcgatgccctcgtgatgacctgcggcttgccacactcaatgttcccgccatcgagatgctgtttgtgtgtatcgtgagcttgccgtagtggtgcctccgtttcctcacgccaccaagccttccccgcagccgagccagctgtgctgagctgtggctgtcgtagagtataaagcctaaatcgcatccgcatcctcgagcagctcatcttctatccatagtccaagcacattgtgtcagattgctcgtcggcatcagagtagctactcgacattcattgagcatatctcgctccgtaccaccaagcccccgagctctactctccattgtcgctgccacgtgtacagtacgtcttgcttttgtctgctcatgggctgtttgccagactgaaccgtgtcgccattagacattctgaccgtaacagcagcccgttagctaccgctccttatcaaaac

SEQ ID NO: 2 - DNA, 840 bp, Trichoderma reesei
  source 1..840: mol_type = genomic DNA
cgtatatgtctatcagtgatgcagctcttaagtcacaaagagatagaattgaacttttgattccaatattagacttcgtattgacggcctactactgaggagcaacttattatagtacgagaacctttggtcgaatcttatgtcttcaagccagatccgggcttgtttcaaggcaccatcttctccccgacttcattacagcccatcaccacatcccccgcacttccatatggaatcacgaatcggaattctcctgttccacgaaatcacatccggcatcatagaaattaatttgtttgcggggtgagtgaccgttcaagttggacaggaagcaaacatcgccaatggcttatacgttcggcatttcccgattaggaaatccggccagcatcagacaacggttgacgagactttgaacacgccagcccaaagcgaatgctctggaatctcgggatctgtccaagaaaagagacaaggcaaaaatgcggagtaactgcttcatcatacaatcacttgcatttatcgatttacagtaaatccggagctcagctcacgagttgcggaggccgaggcggaggcagctaagggggtatcatcaaatccattgttctcgaccacgaaatgatgaacttggatggtggcacaggctcttggatgagatcacgatgatatggaagccttgttttgtctttccgtggtcggagagccccgatgtgggaagatgttgattgtgtaggcctgaatgctgcttatatgccctgctttttgcccttggttattacagtagaattcagacggcacttttattctatccctcaacacattctacagaatagaaca

SEQ ID NO: 3 - DNA, 787 bp, Trichoderma reesei
  source 1..787: mol_type = genomic DNA
tggatgacacggtagacaagcgaatcgaaactttattgttttgttcttgcgttctccctaagtgatgacgaaggaggtgtagcactgaaagtggcagagccacgtacaggagagaacagctcgtacctgatgaactgctgtctcagattgaatatcatacagctcgtggcattgaagctccatagatatgctagcgataagcaggtacagtgaggacacggcttgatcgtggcttgagaatcaccaaggacagtggaacggagtggctgctttggtgattccgaccaactgttcacgagaccagctcggatgcccgggccaacgaatcaaccctccgtaagatggagccacgatcgtataaccctcgctctcaaacagatgttaatatttaggcggaattgtaaactcgggggccctggagaggccgcaactgggcttcatgggcagaacagcggcgccatgccggcatcccagaagtggaatgggcggatcggagctggtgcgcggggggaagtaagctgggtggcaggcccttcggatagctgggagctgtctcaactactagaggagcttagctttggcagctcttgataactgtgacagctattcgccgtttctcgtagtgttcctggactgtgtctgagagctgtcatcccctcatcaccacttacatggacgaacagttgtgtgaatgagcgcaatcatccacctccgttctccatcttcatcatcagccaacatgtccagctcaacgcccacgcggcgcctcatcggcctctcgaccaaa

SEQ ID NO: 4 - DNA, 840 bp, Trichoderma reesei
  source 1..840: mol_type = genomic DNA
tgttctattctgtagaatgtgttgagggatagaataaaagtgccgtctgaattctactgtaataaccaagggcaaaaagcagggcatataagcagcattcaggcctacacaatcaacatcttcccacatcggggctctccgaccacggaaagacaaaacaaggcttccatatcatcgtgatctcatccaagagcctgtgccaccatccaagttcatcatttcgtggtcgagaacaatggatttgatgatacccccttagctgcctccgcctcggcctccgcaactcgtgagctgagctccggatttactgtaaatcgataaatgcaagtgattgtatgatgaagcagttactccgcatttttgccttgtctcttttcttggacagatcccgagattccagagcattcgctttgggctggcgtgttcaaagtctcgtcaaccgttgtctgatgctggccggatttcctaatcgggaaatgccgaacgtataagccattggcgatgtttgcttcctgtccaacttgaacggtcactcaccccgcaaacaaattaatttctatgatgccggatgtgatttcgtggaacaggagaattccgattcgtgattccatatggaagtgcgggggatgtggtgatgggctgtaatgaagtcggggagaagatggtgccttgaaacaagcccggatctggcttgaagacataagattcgaccaaaggttctcgtactataataagttgctcctcagtagtaggccgtcaatacgaagtctaatattggaatcaaaagttcaattctatctctttgtgacttaagagctgcatcactgatagacatatacg

SEQ ID NO: 5 - DNA, 19 bp, synthetic construct
  misc_feature 1..19: note = Primer
  source 1..19: mol_type = other DNA
cggtggtggaagaggattg

SEQ ID NO: 6 - DNA, 20 bp, synthetic construct
  misc_feature 1..20: note = Primer
  source 1..20: mol_type = other DNA
agacggatcaggcaggatgt

SEQ ID NO: 7 - DNA, 20 bp, synthetic construct
  misc_feature 1..20: note = Primer
  source 1..20: mol_type = other DNA
tggacacactcatcccgttt

SEQ ID NO: 8 - DNA, 20 bp, synthetic construct
  misc_feature 1..20: note = Primer
  source 1..20: mol_type = other DNA
ctcttcccagtctcggcttc

SEQ ID NO: 9 - DNA, 20 bp, synthetic construct
  misc_feature 1..20: note = Primer
  source 1..20: mol_type = other DNA
acctgctggagagaagcaca

SEQ ID NO: 10 - DNA, 20 bp, synthetic construct
  misc_feature 1..20: note = Primer
  source 1..20: mol_type = other DNA
ccccatacaaaaccctcgtc

SEQ ID NO: 11 - DNA, 20 bp, synthetic construct
  misc_feature 1..20: note = Primer
  source 1..20: mol_type = other DNA
gtctaggcgtcgccatttct

SEQ ID NO: 12 - DNA, 20 bp, synthetic construct
  misc_feature 1..20: note = Primer
  source 1..20: mol_type = other DNA
caacttccagcccaacaacc

SEQ ID NO: 13 - DNA, 18 bp, synthetic construct
  misc_feature 1..18: note = Primer
  source 1..18: mol_type = other DNA
tctgggcgacatctacat

SEQ ID NO: 14 - DNA, 20 bp, synthetic construct
  misc_feature 1..20: note = Primer
  source 1..20: mol_type = other DNA
gtagtcgagctccttcttca

SEQ ID NO: 15 - DNA, 35 bp, synthetic construct
  misc_feature 1..35: note = Primer
  source 1..35: mol_type = other DNA
attatacgaacggtacttcgacatcaaaatcacct

SEQ ID NO: 16 - DNA, 35 bp, synthetic construct
  misc_feature 1..35: note = Primer
  source 1..35: mol_type = other DNA
gacgtttgctttcatgttttgataaggagcggtag

SEQ ID NO: 17 - DNA, 35 bp, synthetic construct
  misc_feature 1..35: note = Primer
  source 1..35: mol_type = other DNA
attatacgaacggtacgtatatgtctatcagtgat

SEQ ID NO: 18 - DNA, 35 bp, synthetic construct
  misc_feature 1..35: note = Primer
  source 1..35: mol_type = other DNA
gacgtttgctttcattgttctattctgtagaatgt

SEQ ID NO: 19 - DNA, 35 bp, synthetic construct
  misc_feature 1..35: note = Primer
  source 1..35: mol_type = other DNA
attatacgaacggtatggatgacacggtagacaag

SEQ ID NO: 20 - DNA, 35 bp, synthetic construct
  misc_feature 1..35: note = Primer
  source 1..35: mol_type = other DNA
gacgtttgctttcattttggtcgagaggccgatga

SEQ ID NO: 21 - DNA, 35 bp, synthetic construct
  misc_feature 1..35: note = Primer
  source 1..35: mol_type = other DNA
attatacgaacggtatgttctattctgtagaatgt

SEQ ID NO: 22 - DNA, 35 bp, synthetic construct
  misc_feature 1..35: note = Primer
  source 1..35: mol_type = other DNA
gacgtttgctttcatcgtatatgtctatcagtgat

SEQ ID NO: 23 - DNA, 20 bp, synthetic construct
  misc_feature 1..20: note = Primer
  source 1..20: mol_type = other DNA
atgaaagcaaacgtcatctt

SEQ ID NO: 24 - DNA, 35 bp, synthetic construct
  misc_feature 1..35: note = Primer
  source 1..35: mol_type = other DNA
acaacgagaaaagaagtctctggctgagtgctcgt

SEQ ID NO: 25 - DNA, 23 bp, synthetic construct
  misc_feature 1..23: note = Primer
  source 1..23: mol_type = other DNA
ttcttttctcgttgtctcactct

SEQ ID NO: 26 - DNA, 22 bp, synthetic construct
  misc_feature 1..22: note = Primer
  source 1..22: mol_type = other DNA
agatccaccagatatgtcagga